European Patent Specification EP 3 710 595 B1, published September 3, 2025. Title: COMPOSITIONS AND METHODS FOR DETECTING C1orf43 NUCLEIC ACID. Applicant: Gen-Probe Incorporated. The sequence listing filed with the application follows.

SEQUENCE LISTING (72 sequences)

SEQ ID NO: 1 - DNA, 1802 bp, Homo sapiens
gtgcgcgtgccgcctcgccacgagacacctctttccggctccgcgagtccaccccgcctccttcacggcggccctgcctccaccacgtgacgcacggatggccgccgcttcctcttactgtcgtagttccgcgtctgagcgctcgacgctcctgggtgccattgcctgcctgagtcacgtgtcagggggaagctggaaggcgtcgttctcctttcccagctctcctgcctgtccgccatgttttcaggccgggtctggcttggtcttcccccgtaaggaaatggccggggagctccaggggacccaggcgccgtcgcttcggcggagcctgggctgaccagccaggacagcggggtaaacccgaacaattctgcgcgaggtagggaggccatggcgtccggcagtaactggctctccggggtgaatgtcgtgctggtgatggcctacgggagcctggacttgaaagaggagattgatattcgactctccagggttcaggatatcaagtatgagccccagctccttgcagatgatgatgctagactactacaactggaaacccagggaaatcaaagttgctacaactatctgtataggatgaaagctctggatgccattcgtacctctgagatcccatttcattctgaaggccggcatccccgttccttaatgggcaagaatttccgctcctacctgctggatctgcgaaacactagtacgcctttcaagggtgtacgcaaagcactcattgatacccttttggatggctatgaaacagcccgctatgggacaggggtctttggccagaatgagtacctacgctatcaggaggccctgagtgagctggccactgcggttaaagcacgaattgggagctctcagcgacatcaccagtcagcagccaaagacctaactcagtcccctgaggtctccccaacaaccatccaggtgacatacctcccctccagtcagaagagtaaacgtgccaagcacttccttgaattgaagagctttaaggataactataacacattggagagtactctgtgacggagctgaaggactcttgccgtagattaagccagtcagttgcaatgtgcaagacaggctgcttgccgggccgccctcggaacatctggcccagcaggcccagactgtatccatccaagttcccgttgtatccagagttcttagagcttgtgtctaaagggtaattccccaacccttccttatgagcatttttagaacattggctaagactattttcccccagtagcgcttttttctggatttgcattcaggtgttattcttaatgtttctgtcaaagcttcttaaaaatcttcacttggtttcagccatagttcaccttccctgttccaggtttatttaattccaaaggtgagagttggagtgagatgtcttccatatctatacctttgtgcacagttgaatgggaactgtttgggtttagggcatcttagagttgattgatggaaaaagcagacaggaactggtgggaggtcaagtggggaagttggtgaatgtggaataacttacctttgtgctccacttaaaccagatgtgttgcagctttcctgacatgcaaggatctactttaattccacactctcattaataaattgaataaaagggaatgttttggcacctgatataatctgccaggctatgtgacagtaggaaggaatggtttcccctaacaagcccaatgcactggtctgactttataaattatttaataaaatgaactattatcaaataaaacgtatgaatcagtccttta

SEQ ID NO: 2 - skipped

SEQ ID NO: 3 - DNA, 1012 bp, Artificial Sequence
  Construct for in vitro transcription
  MISC_FEATURE (17)..(36): T7 promoter
cgacgaagactctctttaatacgactcactatagggaagcttgtgcgcgtgccgcctcgccacgagacacctctttccggctccgcgagtccaccccgcctccttcacggcggccctgcctccaccacgtgacgcacggatggccgccgcttcctcttactgtcgtagttccgcgtctgagcgctcgacgctcctgggtgccattgcctgcctgagtcacgtgtcagggggaagctggaaggcgtcgttctcctttcccagctctcctgcctgtccgccatgttttcaggccgggtctggcttggtcttcccccgtaaggaaatggccggggagctccaggggacccaggcgccgtcgcttcggcggagcctgggctgaccagccaggacagcggggtaaacccgaacaattctgcgcgaggtagggaggccatggcgtccggcagtaactggctctccggggtgaatgtcgtgctggtgatggcctacgggagcctggacttgaaagaggagattgatattcgactctccagggttcaggatatcaagtatgagccccagctccttgcagatgatgatgctagactactacaactggaaacccagggaaatcaaagttgctacaactatctgtataggatgaaagctctggatgccattcgtacctctgagatcccatttcattctgaaggccggcatccccgttccttaatgggcaagaatttccgctcctacctgctggatctgcgaaacactagtacgcctttcaagggtgtacgcaaagcactcattgatacccttttggatggctatgaaacagcccgctatgggacaggggtctttggccagaatgagtacctacgctatcaggaggccctgagtgagctggccactgcggttaaagcacgaattgggagctctcagcgacatcaccagtcagcagccaaagacctaactcagtcccctgaggtctccccaacaaccatcgcggccgcgtccatccaacacatgc

SEQ ID NO: 4 - DNA, 58 bp, Artificial Sequence
  Capture oligomer
ccaaacagttcccattcaactgtgctttaaaaaaaaaaaaaaaaaaaaaaaaaaaaaa

SEQ ID NO: 5 - DNA, 25 bp, Artificial Sequence
  Capture oligomer THS
ccaaacagttcccattcaactgtgc

SEQ ID NO: 6 - DNA, 60 bp, Artificial Sequence
  Capture oligomer
  misc_feature (1)..(60): N = U
caaaggnanagananggaagacancnctttaaaaaaaaaaaaaaaaaaaaaaaaaaaaaa

SEQ ID NO: 7 - DNA, 27 bp, Artificial Sequence
  Capture oligomer THS
  misc_feature (1)..(27): N = U
caaaggnanagananggaagacancnc

SEQ ID NO: 8 - DNA, 57 bp, Artificial Sequence
  Capture oligomer
  misc_feature (1)..(57): N = U
cngngcacaaaggnanagananggtttaaaaaaaaaaaaaaaaaaaaaaaaaaaaaa

SEQ ID NO: 9 - DNA, 24 bp, Artificial Sequence
  Capture oligomer THS
  misc_feature (1)..(24): N = U
cngngcacaaaggnanaganangg

SEQ ID NO: 10 - DNA, 58 bp, Artificial Sequence
  Capture oligomer
  misc_feature (1)..(58): N = U
canncaacngngcacaaaggnanagtttaaaaaaaaaaaaaaaaaaaaaaaaaaaaaa

SEQ ID NO: 11 - DNA, 25 bp, Artificial Sequence
  Capture oligomer THS
  misc_feature (1)..(25): N = U
canncaacngngcacaaaggnanag

SEQ ID NO: 12 - DNA, 58 bp, Artificial Sequence
  Capture oligomer
  misc_feature (1)..(58): N = U
ccaaacagnncccanncaacngngctttaaaaaaaaaaaaaaaaaaaaaaaaaaaaaa

SEQ ID NO: 13 - DNA, 25 bp, Artificial Sequence
  Capture oligomer THS
  misc_feature (1)..(25): N = U
ccaaacagnncccanncaacngngc

SEQ ID NO: 14 - DNA, 26 bp, Artificial Sequence
  C1orf43 molecular torch. 5F3D.
  misc_feature (1)..(20): N = U
  misc_feature (23)..(24): N = 2'-O-methylated C
  misc_feature (25)..(25): N = 2'-O-methylated A
  misc_feature (26)..(26): N = 2'-O-methylated C
gnggaanaacnnaccnnngngcnnnn

SEQ ID NO: 15 - DNA, 22 bp, Artificial Sequence
  C1orf43 detection oligomer THS
  misc_feature (1)..(22): N = U
gnggaanaacnnaccnnngngc

SEQ ID NO: 16 - DNA, 25 bp, Artificial Sequence
  C1orf43 molecular torch. 21-C9. 5F3D.
  misc_feature (1)..(20): N = U
  misc_feature (21)..(22): (CH2)9-linker follows position 21
  misc_feature (22)..(22): N = 2'-O-methylated G
  misc_feature (23)..(23): N = 2'-O-methylated A
  misc_feature (24)..(25): N = 2'-O-methylated C
ggncaagnggggaagnnggngnnnn

SEQ ID NO: 17 - DNA, 21 bp, Artificial Sequence
  C1orf43 detection oligomer THS
  misc_feature (1)..(21): N = U
ggncaagnggggaagnnggng

SEQ ID NO: 18 - DNA, 23 bp, Artificial Sequence
  C1orf43 molecular torch. 19-C9. 5F3D.
  misc_feature (1)..(17): N = U
  misc_feature (19)..(20): (CH2)9-linker follows position 19
  misc_feature (20)..(20): N = 2'-O-methylated U
  misc_feature (21)..(23): N = 2'-O-methylated C
gggaagnnggngaangnggnnnn

SEQ ID NO: 19 - DNA, 19 bp, Artificial Sequence
  C1orf43 detection oligomer THS
  misc_feature (1)..(19): N = U
gggaagnnggngaangngg

SEQ ID NO: 20 - DNA, 26 bp, Artificial Sequence
  C1orf43 molecular torch. 5F3D.
  misc_feature (1)..(19): N = U
  misc_feature (23)..(23): N = 2'-O-methylated C
  misc_feature (24)..(24): N = 2'-O-methylated A
  misc_feature (25)..(26): N = 2'-O-methylated A
ggngaangnggaanaacnnaccnnnn

SEQ ID NO: 21 - DNA, 22 bp, Artificial Sequence
  C1orf43 detection oligomer THS
  misc_feature (1)..(22): N = U
ggngaangnggaanaacnnacc

SEQ ID NO: 22 - DNA, 32 bp, Artificial Sequence
  C1orf43 molecular beacon. 5F3D.
  misc_feature (1)..(2): N = 2'-O-methylated G
  misc_feature (3)..(3): N = 2'-O-methylated C
  misc_feature (4)..(4): N = 2'-O-methylated U
  misc_feature (5)..(5): N = 2'-O-methylated C
  misc_feature (6)..(25): N = U
  misc_feature (28)..(28): N = 2'-O-methylated G
  misc_feature (29)..(29): N = 2'-O-methylated A
  misc_feature (30)..(30): N = 2'-O-methylated A
  misc_feature (31)..(32): N = 2'-O-methylated C
nnnnngnggaanaacnnaccnnngngcnnnnn

SEQ ID NO: 23 - DNA, 22 bp, Artificial Sequence
  C1orf43 detection oligomer THS
  misc_feature (1)..(22): N = U
gnggaanaacnnaccnnngngc

SEQ ID NO: 24 - DNA, 32 bp, Artificial Sequence
  C1orf43 molecular beacon. 5F3D.
  misc_feature (1)..(2): N = 2'-O-methylated G
  misc_feature (3)..(3): N = 2'-O-methylated C
  misc_feature (4)..(4): N = 2'-O-methylated U
  misc_feature (5)..(5): N = 2'-O-methylated C
  misc_feature (6)..(27): N = U
  misc_feature (28)..(28): N = 2'-O-methylated G
  misc_feature (29)..(29): N = 2'-O-methylated A
  misc_feature (30)..(30): N = 2'-O-methylated G
  misc_feature (31)..(32): N = 2'-O-methylated C
ggcncggngaangnggaanaacnnaccnnnnn

SEQ ID NO: 25 - DNA, 22 bp, Artificial Sequence
  C1orf43 detection oligomer THS
  misc_feature (1)..(22): N = U
ggngaangnggaanaacnnacc

SEQ ID NO: 26 - DNA, 55 bp, Artificial Sequence
  C1orf43 promoter primer
aatttaatacgactcactatagggagagcatgtcaggaaagctgcaacacatctg

SEQ ID NO: 27 - DNA, 28 bp, Artificial Sequence
  C1orf43 amplification oligomer or amplification oligomer THS
gcatgtcaggaaagctgcaacacatctg

SEQ ID NO: 28 - DNA, 55 bp, Artificial Sequence
  C1orf43 promoter primer
aatttaatacgactcactatagggagagctgcaacacatctggtttaagtggagc

SEQ ID NO: 29 - DNA, 28 bp, Artificial Sequence
  C1orf43 amplification oligomer or amplification oligomer THS
gctgcaacacatctggtttaagtggagc

SEQ ID NO: 30 - DNA, 54 bp, Artificial Sequence
  C1orf43 promoter primer
aatttaatacgactcactatagggagaggaaagctgcaacacatctggtttaag

SEQ ID NO: 31 - DNA, 27 bp, Artificial Sequence
  C1orf43 amplification oligomer or amplification oligomer THS
ggaaagctgcaacacatctggtttaag

SEQ ID NO: 32 - DNA, 55 bp, Artificial Sequence
  C1orf43 promoter primer
aatttaatacgactcactatagggagagtagatccttgcatgtcaggaaagctgc

SEQ ID NO: 33 - DNA, 28 bp, Artificial Sequence
  C1orf43 amplification oligomer or amplification oligomer THS
gtagatccttgcatgtcaggaaagctgc

SEQ ID NO: 34 - DNA, 21 bp, Artificial Sequence
  C1orf43 amplification oligomer or amplification oligomer THS
gcagacaggaactggtgggag

SEQ ID NO: 35 - DNA, 23 bp, Artificial Sequence
  C1orf43 amplification oligomer or amplification oligomer THS
ggcatcttagagttgattgatgg

SEQ ID NO: 36 - DNA, 25 bp, Artificial Sequence
  C1orf43 amplification oligomer or amplification oligomer THS
cttagagttgattgatggaaaaagc

SEQ ID NO: 37 - DNA, 21 bp, Artificial Sequence
  C1orf43 amplification oligomer or amplification oligomer THS
ggaaaaagcagacaggaactg

SEQ ID NO: 38 - DNA, 18 bp, Artificial Sequence
  C1orf43 amplification oligomer or amplification oligomer THS
gcagacaggaactggtgg

SEQ ID NO: 39 - DNA, 202 bp, Artificial Sequence
  C1orf43 region encompassing exemplary amplicons
gagatgtcttccatatctatacctttgtgcacagttgaatgggaactgtttgggtttagggcatcttagagttgattgatggaaaaagcagacaggaactggtgggaggtcaagtggggaagttggtgaatgtggaataacttacctttgtgctccacttaaaccagatgtgttgcagctttcctgacatgcaaggatctac

SEQ ID NO: 40 - DNA, 143 bp, Artificial Sequence
  Exemplary C1orf43 amplification product
ggcatcttagagttgattgatggaaaaagcagacaggaactggtgggaggtcaagtggggaagttggtgaatgtggaataacttacctttgtgctccacttaaaccagatgtgttgcagctttcctgacatgcaaggatctac

SEQ ID NO: 41 - DNA, 105 bp, Artificial Sequence
  Exemplary C1orf43 amplification product
gcagacaggaactggtgggaggtcaagtggggaagttggtgaatgtggaataacttacctttgtgctccacttaaaccagatgtgttgcagctttcctgacatgc

SEQ ID NO: 42 - DNA, 92 bp, Artificial Sequence
  Exemplary C1orf43 amplification product
gcagacaggaactggtgggaggtcaagtggggaagttggtgaatgtggaataacttacctttgtgctccacttaaaccagatgtgttgcagc

SEQ ID NO: 43 - DNA, 92 bp, Artificial Sequence
  C1orf43 region encompassing exemplary detection oligomer hybridization sites
aaaaagcagacaggaactggtgggaggtcaagtggggaagttggtgaatgtggaataacttacctttgtgctccacttaaaccagatgtgtt

SEQ ID NO: 44 - DNA, 55 bp, Artificial Sequence
  C1orf43 region encompassing exemplary detection oligomer hybridization sites
tcaagtggggaagttggtgaatgtggaataacttacctttgtgctccacttaaac

SEQ ID NO: 45 - DNA, 43 bp, Artificial Sequence
  C1orf43 region encompassing exemplary detection oligomer hybridization sites
gtcaagtggggaagttggtgaatgtggaataacttacctttgt

SEQ ID NO: 46 - DNA, 49 bp, Artificial Sequence
  C1orf43 region encompassing exemplary amplification oligomer (e.g., nonT7) hybridization sites
ggcatcttagagttgattgatggaaaaagcagacaggaactggtgggag

SEQ ID NO: 47 - DNA, 14 bp, Artificial Sequence
  exemplary amplification oligomer (e.g., nonT7) core sequence
gcagacaggaactg

SEQ ID NO: 48 - DNA, 18 bp, Artificial Sequence
  exemplary amplification oligomer (e.g., nonT7) core sequence
cttagagttgattgatgg

SEQ ID NO: 49 - DNA, 46 bp, Artificial Sequence
  C1orf43 region encompassing exemplary detection oligomer hybridization sites
  misc_feature (1)..(46): N = U
ggncaagnggggaagnnggngaangnggaanaacnnaccnnngngc

SEQ ID NO: 50 - DNA, 15 bp, Artificial Sequence
  exemplary detection oligomer core seqeunce
  misc_feature (1)..(15): N = U
gnggaanaacnnacc

SEQ ID NO: 51 - DNA, 13 bp, Artificial Sequence
  exemplary detection oligomer core seqeunce
  misc_feature (1)..(13): N = U
ggggaagnnggng

SEQ ID NO: 52 - DNA, 51 bp, Artificial Sequence
  C1orf43 region encompassing exemplary amplification oligomer (e.g., promoter primer) hybridization sites
  misc-feature (1)..(51): N = U
gtagatccttgcatgtcaggaaagctgcaacacatctggtttaagtggagc

SEQ ID NO: 53 - DNA, 15 bp, Artificial Sequence
  Exemplary amplification oligomer (e.g., promoter primer) core sequence
gctgcaacacatctg

SEQ ID NO: 54 - DNA, 10 bp, Artificial Sequence
  Exemplary amplification oligomer (e.g., promoter primer) core sequence
ggaaagctgc

SEQ ID NO: 55 - DNA, 53 bp, Artificial Sequence
  C1orf43 region encompassing exemplary capture oligomer hybridization sites
  misc_feature (1)..(53): N = U
ccaaacagnncccanncaacngngcacaaaggnanagananggaagacancnc

SEQ ID NO: 56 - DNA, 11 bp, Artificial Sequence
  Exemplary capture oligomer core sequence
  misc_feature (1)..(11): N = U
caaaggnanag

SEQ ID NO: 57 - DNA, 13 bp, Artificial Sequence
  Exemplary capture oligomer core sequence
  misc_feature (1)..(13): N = U
canncaacngngc

SEQ ID NO: 58 - DNA, 27 bp, Artificial Sequence
  Exemplary T7 promoter sequence
  misc_feature (1)..(27): N = U
aatttaatacgactcactatagggaga

SEQ ID NO: 59 - DNA, 20 bp, Artificial Sequence
  C1orf43 linear detection probe
  misc_feature (1)..(20): N = U
gngaangnggaanaacnnac

SEQ ID NO: 60 - DNA, 15 bp, Artificial Sequence
  C1orf43 linear detection probe
  misc_feature (1)..(15): N = U
gnggggaagnnggng

SEQ ID NO: 61 - DNA, 19 bp, Artificial Sequence
  C1orf43 linear detection probe
  misc_feature (1)..(19): N = U
caccnnanngaanggaaac

SEQ ID NO: 62 - DNA, 17 bp, Artificial Sequence
  C1orf43 linear detection probe
  misc_feature (1)..(17): N = U
cnncaaccacnnacacc

SEQ ID NO: 63 - DNA, 19 bp, Artificial Sequence
  C1orf43 linear detection probe
  misc_feature (1)..(19): N = U
cnnacaccnnanngaangg

SEQ ID NO: 64 - DNA, 18 bp, Artificial Sequence
  C1orf43 linear detection probe
  misc_feature (1)..(18): N = U
gaanaacnnaccnnngng

SEQ ID NO: 65 - DNA, 20 bp, Artificial Sequence
  C1orf43 linear detection probe
  misc_feature (1)..(20): N = U
caaccacnnacaccnnanng

SEQ ID NO: 66 - DNA, 16 bp, Artificial Sequence
  C1orf43 linear detection probe
  misc_feature (1)..(16): N = U
gaagnnggngaangng

SEQ ID NO: 67 - DNA, 19 bp, Artificial Sequence
  C1orf43 linear detection probe
  misc_feature (1)..(19): N = U
gnggaanaacnnaccnnng

SEQ ID NO: 68 - DNA, 19 bp, Artificial Sequence
  C1orf43 linear detection probe
  misc_feature (1)..(19): N = U
gnggggaagnnggngaang

SEQ ID NO: 69 - DNA, 14 bp, Artificial Sequence
  C1orf43 linear detection probe
  misc_feature (1)..(14): N = U
gaangnggaanaac

SEQ ID NO: 70 - DNA, 18 bp, Artificial Sequence
  C1orf43 linear detection probe
  misc_feature (1)..(18): N = U
cnnaccnnngngcnccac

SEQ ID NO: 71 - DNA, 21 bp, Artificial Sequence
  C1orf43 linear detection probe
  misc_feature (1)..(21): N = U
gaanaacnnaccnnngngcnc

SEQ ID NO: 72 - DNA, 17 bp, Artificial Sequence
  C1orf43 linear detection probe
  misc_feature (1)..(17): N = U
gncaagnggggaagnng